European Patent Specification EP 2 952 587 B1, published July 5, 2023. Title: HIGH THROUGHPUT NUCLEIC ACID SEQUENCING BY EXPANSION. Applicant: STRATOS GENOMICS INC. Application not yet assigned. The sequence listing filed with the application follows.

SEQUENCE LISTING (6 sequences)

SEQ ID NO: 1 - DNA, 12 bp, Artificial Sequence
  Three Xprobes encode entire contiguous sequence
actggccgaaat

SEQ ID NO: 2 - DNA, 36 bp, Artificial Sequence
  Synthesized template sequence
tgtgtgtgtgtgtgtgtgtgatctaccgtccgtccc

SEQ ID NO: 3 - DNA, 16 bp, Artificial Sequence
  Primer
gggacggacggtagat

SEQ ID NO: 4 - DNA, 32 bp, Artificial Sequence
  Synthesized template sequence
tctctctctctctctcatctaccgtccgtccc

SEQ ID NO: 5 - protein, 49 aa, Artificial Sequence
  Synthesized peptide on a solid support
ECGAGAGAGAGAGAGAGAGAGAPSGSPAGAGAGAGAGAGAGAGAGAGCK

SEQ ID NO: 6 - DNA, 36 bp, Artificial Sequence
  Synthesized template sequence
ttttttttttttttttttttatctaccgtccgtccc